European Patent Application EP 4 450 515 A1, published October 23, 2024. Title: 突变的蛋白A结构域C及其应用. Applicant: 博格隆（上海）生物技术有限公司. The sequence listing filed with the application follows.

SEQUENCE LISTING (109 sequences)

SEQ ID NO: 1 - protein, 58 aa, synthetic construct
ADNKFNKEQQNAFYEILHLPNLTEEQRNGFIQSLKDDPSVSKEILAEAKKLNDAQAPK

SEQ ID NO: 2 - protein, 58 aa, synthetic construct
ADLKFNKEQQNAFYEILHLPNLTEEQRNGFIQSLKDDPSVSKEILAEAKKLNDAQAPK

SEQ ID NO: 3 - protein, 58 aa, synthetic construct
ADVKFNKEQQNAFYEILHLPNLTEEQRNGFIQSLKDDPSVSKEILAEAKKLNDAQAPK

SEQ ID NO: 4 - protein, 58 aa, synthetic construct
ADYKFNKEQQNAFYEILHLPNLTEEQRNGFIQSLKDDPSVSKEILAEAKKLNDAQAPK

SEQ ID NO: 5 - protein, 58 aa, synthetic construct
ADNKFSKEQQNAFYEILHLPNLTEEQRNGFIQSLKDDPSVSKEILAEAKKLNDAQAPK

SEQ ID NO: 6 - protein, 58 aa, synthetic construct
ADNKFLKEQQNAFYEILHLPNLTEEQRNGFIQSLKDDPSVSKEILAEAKKLNDAQAPK

SEQ ID NO: 7 - protein, 58 aa, synthetic construct
ADNKFEKEQQNAFYEILHLPNLTEEQRNGFIQSLKDDPSVSKEILAEAKKLNDAQAPK

SEQ ID NO: 8 - protein, 58 aa, synthetic construct
ADNKFNKEIQNAFYEILHLPNLTEEQRNGFIQSLKDDPSVSKEILAEAKKLNDAQAPK

SEQ ID NO: 9 - protein, 58 aa, synthetic construct
ADNKFNKEFQNAFYEILHLPNLTEEQRNGFIQSLKDDPSVSKEILAEAKKLNDAQAPK

SEQ ID NO: 10 - protein, 58 aa, synthetic construct
ADNKFNKEMQNAFYEILHLPNLTEEQRNGFIQSLKDDPSVSKEILAEAKKLNDAQAPK

SEQ ID NO: 11 - protein, 58 aa, synthetic construct
ADNKFNKEQQNAFYTILHLPNLTEEQRNGFIQSLKDDPSVSKEILAEAKKLNDAQAPK

SEQ ID NO: 12 - protein, 58 aa, synthetic construct
ADNKFNKEQQNAFYWILHLPNLTEEQRNGFIQSLKDDPSVSKEILAEAKKLNDAQAPK

SEQ ID NO: 13 - protein, 58 aa, synthetic construct
ADNKFNKEQQNAFYLILHLPNLTEEQRNGFIQSLKDDPSVSKEILAEAKKLNDAQAPK

SEQ ID NO: 14 - protein, 58 aa, synthetic construct
ADNKFNKEQQNAFYVILHLPNLTEEQRNGFIQSLKDDPSVSKEILAEAKKLNDAQAPK

SEQ ID NO: 15 - protein, 58 aa, synthetic construct
ADNKFNKEQQNAFYIILHLPNLTEEQRNGFIQSLKDDPSVSKEILAEAKKLNDAQAPK

SEQ ID NO: 16 - protein, 58 aa, synthetic construct
ADNKFNKEQQNAFYFILHLPNLTEEQRNGFIQSLKDDPSVSKEILAEAKKLNDAQAPK

SEQ ID NO: 17 - protein, 58 aa, synthetic construct
ADNKFNKEQQNAFYSILHLPNLTEEQRNGFIQSLKDDPSVSKEILAEAKKLNDAQAPK

SEQ ID NO: 18 - protein, 58 aa, synthetic construct
ADNKFNKEQQNAFYYILHLPNLTEEQRNGFIQSLKDDPSVSKEILAEAKKLNDAQAPK

SEQ ID NO: 19 - protein, 58 aa, synthetic construct
ADNKFNKEQQNAFYDILHLPNLTEEQRNGFIQSLKDDPSVSKEILAEAKKLNDAQAPK

SEQ ID NO: 20 - protein, 58 aa, synthetic construct
ADNKFNKEIQNAFYTILHLPNLTEEQRNGFIQSLKDDPSVSKEILAEAKKLNDAQAPK

SEQ ID NO: 21 - protein, 58 aa, synthetic construct
ADNKFNKEIQNAFYWILHLPNLTEEQRNGFIQSLKDDPSVSKEILAEAKKLNDAQAPK

SEQ ID NO: 22 - protein, 58 aa, synthetic construct
ADNKFNKEIQNAFYLILHLPNLTEEQRNGFIQSLKDDPSVSKEILAEAKKLNDAQAPK

SEQ ID NO: 23 - protein, 58 aa, synthetic construct
ADNKFNKEIQNAFYVILHLPNLTEEQRNGFIQSLKDDPSVSKEILAEAKKLNDAQAPK

SEQ ID NO: 24 - protein, 58 aa, synthetic construct
ADNKFNKEIQNAFYIILHLPNLTEEQRNGFIQSLKDDPSVSKEILAEAKKLNDAQAPK

SEQ ID NO: 25 - protein, 58 aa, synthetic construct
ADNKFNKEIQNAFYFILHLPNLTEEQRNGFIQSLKDDPSVSKEILAEAKKLNDAQAPK

SEQ ID NO: 26 - protein, 58 aa, synthetic construct
ADNKFNKEIQNAFYSILHLPNLTEEQRNGFIQSLKDDPSVSKEILAEAKKLNDAQAPK

SEQ ID NO: 27 - protein, 58 aa, synthetic construct
ADNKFNKEIQNAFYYILHLPNLTEEQRNGFIQSLKDDPSVSKEILAEAKKLNDAQAPK

SEQ ID NO: 28 - protein, 58 aa, synthetic construct
ADNKFNKEIQNAFYDILHLPNLTEEQRNGFIQSLKDDPSVSKEILAEAKKLNDAQAPK

SEQ ID NO: 29 - protein, 58 aa, synthetic construct
ADNKFNKEFQNAFYTILHLPNLTEEQRNGFIQSLKDDPSVSKEILAEAKKLNDAQAPK

SEQ ID NO: 30 - protein, 58 aa, synthetic construct
ADNKFNKEFQNAFYWILHLPNLTEEQRNGFIQSLKDDPSVSKEILAEAKKLNDAQAPK

SEQ ID NO: 31 - protein, 58 aa, synthetic construct
ADNKFNKEFQNAFYLILHLPNLTEEQRNGFIQSLKDDPSVSKEILAEAKKLNDAQAPK

SEQ ID NO: 32 - protein, 58 aa, synthetic construct
ADNKFNKEFQNAFYVILHLPNLTEEQRNGFIQSLKDDPSVSKEILAEAKKLNDAQAPK

SEQ ID NO: 33 - protein, 58 aa, synthetic construct
ADNKFNKEFQNAFYIILHLPNLTEEQRNGFIQSLKDDPSVSKEILAEAKKLNDAQAPK

SEQ ID NO: 34 - protein, 58 aa, synthetic construct
ADNKFNKEFQNAFYFILHLPNLTEEQRNGFIQSLKDDPSVSKEILAEAKKLNDAQAPK

SEQ ID NO: 35 - protein, 58 aa, synthetic construct
ADNKFNKEFQNAFYSILHLPNLTEEQRNGFIQSLKDDPSVSKEILAEAKKLNDAQAPK

SEQ ID NO: 36 - protein, 58 aa, synthetic construct
ADNKFNKEFQNAFYYILHLPNLTEEQRNGFIQSLKDDPSVSKEILAEAKKLNDAQAPK

SEQ ID NO: 37 - protein, 58 aa, synthetic construct
ADNKFNKEFQNAFYDILHLPNLTEEQRNGFIQSLKDDPSVSKEILAEAKKLNDAQAPK

SEQ ID NO: 38 - protein, 58 aa, synthetic construct
ADLKFNKEIQNAFYWILHLPNLTEEQRNGFIQSLKDDPSVSKEILAEAKKLNDAQAPK

SEQ ID NO: 39 - protein, 58 aa, synthetic construct
ADLKFNKEIQNAFYLILHLPNLTEEQRNGFIQSLKDDPSVSKEILAEAKKLNDAQAPK

SEQ ID NO: 40 - protein, 58 aa, synthetic construct
ADLKFNKEIQNAFYVILHLPNLTEEQRNGFIQSLKDDPSVSKEILAEAKKLNDAQAPK

SEQ ID NO: 41 - protein, 58 aa, synthetic construct
ADLKFNKEIQNAFYIILHLPNLTEEQRNGFIQSLKDDPSVSKEILAEAKKLNDAQAPK

SEQ ID NO: 42 - protein, 58 aa, synthetic construct
ADLKFNKEIQNAFYFILHLPNLTEEQRNGFIQSLKDDPSVSKEILAEAKKLNDAQAPK

SEQ ID NO: 43 - protein, 58 aa, synthetic construct
ADVKFNKEIQNAFYWILHLPNLTEEQRNGFIQSLKDDPSVSKEILAEAKKLNDAQAPK

SEQ ID NO: 44 - protein, 58 aa, synthetic construct
ADVKFNKEIQNAFYLILHLPNLTEEQRNGFIQSLKDDPSVSKEILAEAKKLNDAQAPK

SEQ ID NO: 45 - protein, 58 aa, synthetic construct
ADVKFNKEIQNAFYVILHLPNLTEEQRNGFIQSLKDDPSVSKEILAEAKKLNDAQAPK

SEQ ID NO: 46 - protein, 58 aa, synthetic construct
ADVKFNKEIQNAFYIILHLPNLTEEQRNGFIQSLKDDPSVSKEILAEAKKLNDAQAPK

SEQ ID NO: 47 - protein, 58 aa, synthetic construct
ADVKFNKEIQNAFYFILHLPNLTEEQRNGFIQSLKDDPSVSKEILAEAKKLNDAQAPK

SEQ ID NO: 48 - protein, 58 aa, synthetic construct
ADNKFLKEFQNAFYWILHLPNLTEEQRNGFIQSLKDDPSVSKEILAEAKKLNDAQAPK

SEQ ID NO: 49 - protein, 58 aa, synthetic construct
ADNKFLKEFQNAFYLILHLPNLTEEQRNGFIQSLKDDPSVSKEILAEAKKLNDAQAPK

SEQ ID NO: 50 - protein, 58 aa, synthetic construct
ADNKFLKEFQNAFYVILHLPNLTEEQRNGFIQSLKDDPSVSKEILAEAKKLNDAQAPK

SEQ ID NO: 51 - protein, 58 aa, synthetic construct
ADNKFLKEFQNAFYIILHLPNLTEEQRNGFIQSLKDDPSVSKEILAEAKKLNDAQAPK

SEQ ID NO: 52 - protein, 58 aa, synthetic construct
ADNKFLKEFQNAFYFILHLPNLTEEQRNGFIQSLKDDPSVSKEILAEAKKLNDAQAPK

SEQ ID NO: 53 - protein, 58 aa, synthetic construct
ADNKFEKEFQNAFYWILHLPNLTEEQRNGFIQSLKDDPSVSKEILAEAKKLNDAQAPK

SEQ ID NO: 54 - protein, 58 aa, synthetic construct
ADNKFEKEFQNAFYLILHLPNLTEEQRNGFIQSLKDDPSVSKEILAEAKKLNDAQAPK

SEQ ID NO: 55 - protein, 58 aa, synthetic construct
ADNKFEKEFQNAFYVILHLPNLTEEQRNGFIQSLKDDPSVSKEILAEAKKLNDAQAPK

SEQ ID NO: 56 - protein, 58 aa, synthetic construct
ADNKFEKEFQNAFYIILHLPNLTEEQRNGFIQSLKDDPSVSKEILAEAKKLNDAQAPK

SEQ ID NO: 57 - protein, 58 aa, synthetic construct
ADNKFEKEFQNAFYFILHLPNLTEEQRNGFIQSLKDDPSVSKEILAEAKKLNDAQAPK

SEQ ID NO: 58 - protein, 58 aa, synthetic construct
ADLKFLKEIQNAFYWILHLPNLTEEQRNGFIQSLKDDPSVSKEILAEAKKLNDAQAPK

SEQ ID NO: 59 - protein, 58 aa, synthetic construct
ADLKFLKEIQNAFYLILHLPNLTEEQRNGFIQSLKDDPSVSKEILAEAKKLNDAQAPK

SEQ ID NO: 60 - protein, 58 aa, synthetic construct
ADYKFEKEIQNAFYLILHLPNLTEEQRNGFIQSLKDDPSVSKEILAEAKKLNDAQAPK

SEQ ID NO: 61 - protein, 58 aa, synthetic construct
ADYKFEKEIQNAFYIILHLPNLTEEQRNGFIQSLKDDPSVSKEILAEAKKLNDAQAPK

SEQ ID NO: 62 - protein, 58 aa, synthetic construct
ADVKFLKEIQNAFYVILHLPNLTEEQRNGFIQSLKDDPSVSKEILAEAKKLNDAQAPK

SEQ ID NO: 63 - protein, 58 aa, synthetic construct
ADVKFEKEIQNAFYLILHLPNLTEEQRNGFIQSLKDDPSVSKEILAEAKKLNDAQAPK

SEQ ID NO: 64 - protein, 58 aa, synthetic construct
ADVKFEKEIQNAFYIILHLPNLTEEQRNGFIQSLKDDPSVSKEILAEAKKLNDAQAPK

SEQ ID NO: 65 - protein, 58 aa, synthetic construct
ADVKFEKEIQNAFYFILHLPNLTEEQRNGFIQSLKDDPSVSKEILAEAKKLNDAQAPK

SEQ ID NO: 66 - protein, 58 aa, synthetic construct
ADLKFLKEFQNAFYWILHLPNLTEEQRNGFIQSLKDDPSVSKEILAEAKKLNDAQAPK

SEQ ID NO: 67 - protein, 58 aa, synthetic construct
ADLKFLKEFQNAFYIILHLPNLTEEQRNGFIQSLKDDPSVSKEILAEAKKLNDAQAPK

SEQ ID NO: 68 - protein, 58 aa, synthetic construct
ADLKFEKEFQNAFYLILHLPNLTEEQRNGFIQSLKDDPSVSKEILAEAKKLNDAQAPK

SEQ ID NO: 69 - protein, 58 aa, synthetic construct
ADVKFLKEFQNAFYVILHLPNLTEEQRNGFIQSLKDDPSVSKEILAEAKKLNDAQAPK

SEQ ID NO: 70 - protein, 58 aa, synthetic construct
ADVKFEKEFQNAFYIILHLPNLTEEQRNGFIQSLKDDPSVSKEILAEAKKLNDAQAPK

SEQ ID NO: 71 - protein, 58 aa, synthetic construct
ADVKFEKEFQNAFYFILHLPNLTEEQRNGFIQSLKDDPSVSKEILAEAKKLNDAQAPK

SEQ ID NO: 72 - protein, 58 aa, synthetic construct
ADLKFEKEFQNAFYIILHLPNLTEEQRNGFIQSLKDDPSVSKEILAEAKKLNDAQAPK

SEQ ID NO: 73 - protein, 58 aa, synthetic construct
ADVKFLKEFQNAFYLILHLPNLTEEQRNGFIQSLKDDPSVSKEILAEAKKLNDAQAPK

SEQ ID NO: 74 - protein, 232 aa, synthetic construct
ADNKFNKEQQNAFYEILHLPNLTEEQRNGFIQSLKDDPSVSKEILAEAKKLNDAQAPKADNKFNKEQQNAFYEILHLPNLTEEQRNGFIQSLKDDPSVSKEILAEAKKLNDAQAPKADNKFNKEQQNAFYEILHLPNLTEEQRNGFIQSLKDDPSVSKEILAEAKKLNDAQAPKADNKFNKEQQNAFYEILHLPNLTEEQRNGFIQSLKDDPSVSKEILAEAKKLNDAQAPK

SEQ ID NO: 75 - protein, 232 aa, synthetic construct
ADLKFNKEQQNAFYEILHLPNLTEEQRNGFIQSLKDDPSVSKEILAEAKKLNDAQAPKADLKFNKEQQNAFYEILHLPNLTEEQRNGFIQSLKDDPSVSKEILAEAKKLNDAQAPKADLKFNKEQQNAFYEILHLPNLTEEQRNGFIQSLKDDPSVSKEILAEAKKLNDAQAPKADLKFNKEQQNAFYEILHLPNLTEEQRNGFIQSLKDDPSVSKEILAEAKKLNDAQAPK

SEQ ID NO: 76 - protein, 232 aa, synthetic construct
ADVKFNKEQQNAFYEILHLPNLTEEQRNGFIQSLKDDPSVSKEILAEAKKLNDAQAPKADVKFNKEQQNAFYEILHLPNLTEEQRNGFIQSLKDDPSVSKEILAEAKKLNDAQAPKADVKFNKEQQNAFYEILHLPNLTEEQRNGFIQSLKDDPSVSKEILAEAKKLNDAQAPKADVKFNKEQQNAFYEILHLPNLTEEQRNGFIQSLKDDPSVSKEILAEAKKLNDAQAPK

SEQ ID NO: 77 - protein, 232 aa, synthetic construct
ADNKFLKEQQNAFYEILHLPNLTEEQRNGFIQSLKDDPSVSKEILAEAKKLNDAQAPKADNKFLKEQQNAFYEILHLPNLTEEQRNGFIQSLKDDPSVSKEILAEAKKLNDAQAPKADNKFLKEQQNAFYEILHLPNLTEEQRNGFIQSLKDDPSVSKEILAEAKKLNDAQAPKADNKFLKEQQNAFYEILHLPNLTEEQRNGFIQSLKDDPSVSKEILAEAKKLNDAQAPK

SEQ ID NO: 78 - protein, 232 aa, synthetic construct
ADNKFEKEQQNAFYEILHLPNLTEEQRNGFIQSLKDDPSVSKEILAEAKKLNDAQAPKADNKFEKEQQNAFYEILHLPNLTEEQRNGFIQSLKDDPSVSKEILAEAKKLNDAQAPKADNKFEKEQQNAFYEILHLPNLTEEQRNGFIQSLKDDPSVSKEILAEAKKLNDAQAPKADNKFEKEQQNAFYEILHLPNLTEEQRNGFIQSLKDDPSVSKEILAEAKKLNDAQAPK

SEQ ID NO: 79 - protein, 232 aa, synthetic construct
ADNKFNKEIQNAFYEILHLPNLTEEQRNGFIQSLKDDPSVSKEILAEAKKLNDAQAPKADNKFNKEIQNAFYEILHLPNLTEEQRNGFIQSLKDDPSVSKEILAEAKKLNDAQAPKADNKFNKEIQNAFYEILHLPNLTEEQRNGFIQSLKDDPSVSKEILAEAKKLNDAQAPKADNKFNKEIQNAFYEILHLPNLTEEQRNGFIQSLKDDPSVSKEILAEAKKLNDAQAPK

SEQ ID NO: 80 - protein, 232 aa, synthetic construct
ADNKFNKEFQNAFYEILHLPNLTEEQRNGFIQSLKDDPSVSKEILAEAKKLNDAQAPKADNKFNKEFQNAFYEILHLPNLTEEQRNGFIQSLKDDPSVSKEILAEAKKLNDAQAPKADNKFNKEFQNAFYEILHLPNLTEEQRNGFIQSLKDDPSVSKEILAEAKKLNDAQAPKADNKFNKEFQNAFYEILHLPNLTEEQRNGFIQSLKDDPSVSKEILAEAKKLNDAQAPK

SEQ ID NO: 81 - protein, 232 aa, synthetic construct
ADNKFNKEMQNAFYEILHLPNLTEEQRNGFIQSLKDDPSVSKEILAEAKKLNDAQAPKADNKFNKEMQNAFYEILHLPNLTEEQRNGFIQSLKDDPSVSKEILAEAKKLNDAQAPKADNKFNKEMQNAFYEILHLPNLTEEQRNGFIQSLKDDPSVSKEILAEAKKLNDAQAPKADNKFNKEMQNAFYEILHLPNLTEEQRNGFIQSLKDDPSVSKEILAEAKKLNDAQAPK

SEQ ID NO: 82 - protein, 232 aa, synthetic construct
ADNKFNKEQQNAFYTILHLPNLTEEQRNGFIQSLKDDPSVSKEILAEAKKLNDAQAPKADNKFNKEQQNAFYTILHLPNLTEEQRNGFIQSLKDDPSVSKEILAEAKKLNDAQAPKADNKFNKEQQNAFYTILHLPNLTEEQRNGFIQSLKDDPSVSKEILAEAKKLNDAQAPKADNKFNKEQQNAFYTILHLPNLTEEQRNGFIQSLKDDPSVSKEILAEAKKLNDAQAPK

SEQ ID NO: 83 - protein, 232 aa, synthetic construct
ADNKFNKEQQNAFYWILHLPNLTEEQRNGFIQSLKDDPSVSKEILAEAKKLNDAQAPKADNKFNKEQQNAFYWILHLPNLTEEQRNGFIQSLKDDPSVSKEILAEAKKLNDAQAPKADNKFNKEQQNAFYWILHLPNLTEEQRNGFIQSLKDDPSVSKEILAEAKKLNDAQAPKADNKFNKEQQNAFYWILHLPNLTEEQRNGFIQSLKDDPSVSKEILAEAKKLNDAQAPK

SEQ ID NO: 84 - protein, 232 aa, synthetic construct
ADNKFNKEQQNAFYLILHLPNLTEEQRNGFIQSLKDDPSVSKEILAEAKKLNDAQAPKADNKFNKEQQNAFYLILHLPNLTEEQRNGFIQSLKDDPSVSKEILAEAKKLNDAQAPKADNKFNKEQQNAFYLILHLPNLTEEQRNGFIQSLKDDPSVSKEILAEAKKLNDAQAPKADNKFNKEQQNAFYLILHLPNLTEEQRNGFIQSLKDDPSVSKEILAEAKKLNDAQAPK

SEQ ID NO: 85 - protein, 232 aa, synthetic construct
ADNKFNKEQQNAFYVILHLPNLTEEQRNGFIQSLKDDPSVSKEILAEAKKLNDAQAPKADNKFNKEQQNAFYVILHLPNLTEEQRNGFIQSLKDDPSVSKEILAEAKKLNDAQAPKADNKFNKEQQNAFYVILHLPNLTEEQRNGFIQSLKDDPSVSKEILAEAKKLNDAQAPKADNKFNKEQQNAFYVILHLPNLTEEQRNGFIQSLKDDPSVSKEILAEAKKLNDAQAPK

SEQ ID NO: 86 - protein, 232 aa, synthetic construct
ADNKFNKEQQNAFYIILHLPNLTEEQRNGFIQSLKDDPSVSKEILAEAKKLNDAQAPKADNKFNKEQQNAFYIILHLPNLTEEQRNGFIQSLKDDPSVSKEILAEAKKLNDAQAPKADNKFNKEQQNAFYIILHLPNLTEEQRNGFIQSLKDDPSVSKEILAEAKKLNDAQAPKADNKFNKEQQNAFYIILHLPNLTEEQRNGFIQSLKDDPSVSKEILAEAKKLNDAQAPK

SEQ ID NO: 87 - protein, 232 aa, synthetic construct
ADNKFNKEQQNAFYFILHLPNLTEEQRNGFIQSLKDDPSVSKEILAEAKKLNDAQAPKADNKFNKEQQNAFYFILHLPNLTEEQRNGFIQSLKDDPSVSKEILAEAKKLNDAQAPKADNKFNKEQQNAFYFILHLPNLTEEQRNGFIQSLKDDPSVSKEILAEAKKLNDAQAPKADNKFNKEQQNAFYFILHLPNLTEEQRNGFIQSLKDDPSVSKEILAEAKKLNDAQAPK

SEQ ID NO: 88 - protein, 232 aa, synthetic construct
ADNKFNKEQQNAFYSILHLPNLTEEQRNGFIQSLKDDPSVSKEILAEAKKLNDAQAPKADNKFNKEQQNAFYSILHLPNLTEEQRNGFIQSLKDDPSVSKEILAEAKKLNDAQAPKADNKFNKEQQNAFYSILHLPNLTEEQRNGFIQSLKDDPSVSKEILAEAKKLNDAQAPKADNKFNKEQQNAFYSILHLPNLTEEQRNGFIQSLKDDPSVSKEILAEAKKLNDAQAPK

SEQ ID NO: 89 - protein, 232 aa, synthetic construct
ADNKFNKEQQNAFYYILHLPNLTEEQRNGFIQSLKDDPSVSKEILAEAKKLNDAQAPKADNKFNKEQQNAFYYILHLPNLTEEQRNGFIQSLKDDPSVSKEILAEAKKLNDAQAPKADNKFNKEQQNAFYYILHLPNLTEEQRNGFIQSLKDDPSVSKEILAEAKKLNDAQAPKADNKFNKEQQNAFYYILHLPNLTEEQRNGFIQSLKDDPSVSKEILAEAKKLNDAQAPK

SEQ ID NO: 90 - protein, 232 aa, synthetic construct
ADNKFNKEQQNAFYDILHLPNLTEEQRNGFIQSLKDDPSVSKEILAEAKKLNDAQAPKADNKFNKEQQNAFYDILHLPNLTEEQRNGFIQSLKDDPSVSKEILAEAKKLNDAQAPKADNKFNKEQQNAFYDILHLPNLTEEQRNGFIQSLKDDPSVSKEILAEAKKLNDAQAPKADNKFNKEQQNAFYDILHLPNLTEEQRNGFIQSLKDDPSVSKEILAEAKKLNDAQAPK

SEQ ID NO: 91 - protein, 232 aa, synthetic construct
ADNKFNKEIQNAFYWILHLPNLTEEQRNGFIQSLKDDPSVSKEILAEAKKLNDAQAPKADNKFNKEIQNAFYWILHLPNLTEEQRNGFIQSLKDDPSVSKEILAEAKKLNDAQAPKADNKFNKEIQNAFYWILHLPNLTEEQRNGFIQSLKDDPSVSKEILAEAKKLNDAQAPKADNKFNKEIQNAFYWILHLPNLTEEQRNGFIQSLKDDPSVSKEILAEAKKLNDAQAPK

SEQ ID NO: 92 - protein, 232 aa, synthetic construct
ADNKFNKEIQNAFYLILHLPNLTEEQRNGFIQSLKDDPSVSKEILAEAKKLNDAQAPKADNKFNKEIQNAFYLILHLPNLTEEQRNGFIQSLKDDPSVSKEILAEAKKLNDAQAPKADNKFNKEIQNAFYLILHLPNLTEEQRNGFIQSLKDDPSVSKEILAEAKKLNDAQAPKADNKFNKEIQNAFYLILHLPNLTEEQRNGFIQSLKDDPSVSKEILAEAKKLNDAQAPK

SEQ ID NO: 93 - protein, 232 aa, synthetic construct
ADNKFNKEIQNAFYVILHLPNLTEEQRNGFIQSLKDDPSVSKEILAEAKKLNDAQAPKADNKFNKEIQNAFYVILHLPNLTEEQRNGFIQSLKDDPSVSKEILAEAKKLNDAQAPKADNKFNKEIQNAFYVILHLPNLTEEQRNGFIQSLKDDPSVSKEILAEAKKLNDAQAPKADNKFNKEIQNAFYVILHLPNLTEEQRNGFIQSLKDDPSVSKEILAEAKKLNDAQAPK

SEQ ID NO: 94 - protein, 232 aa, synthetic construct
ADNKFNKEIQNAFYIILHLPNLTEEQRNGFIQSLKDDPSVSKEILAEAKKLNDAQAPKADNKFNKEIQNAFYIILHLPNLTEEQRNGFIQSLKDDPSVSKEILAEAKKLNDAQAPKADNKFNKEIQNAFYIILHLPNLTEEQRNGFIQSLKDDPSVSKEILAEAKKLNDAQAPKADNKFNKEIQNAFYIILHLPNLTEEQRNGFIQSLKDDPSVSKEILAEAKKLNDAQAPK

SEQ ID NO: 95 - protein, 232 aa, synthetic construct
ADNKFNKEIQNAFYFILHLPNLTEEQRNGFIQSLKDDPSVSKEILAEAKKLNDAQAPKADNKFNKEIQNAFYFILHLPNLTEEQRNGFIQSLKDDPSVSKEILAEAKKLNDAQAPKADNKFNKEIQNAFYFILHLPNLTEEQRNGFIQSLKDDPSVSKEILAEAKKLNDAQAPKADNKFNKEIQNAFYFILHLPNLTEEQRNGFIQSLKDDPSVSKEILAEAKKLNDAQAPK

SEQ ID NO: 96 - protein, 232 aa, synthetic construct
ADLKFLKEIQNAFYWILHLPNLTEEQRNGFIQSLKDDPSVSKEILAEAKKLNDAQAPKADLKFLKEIQNAFYWILHLPNLTEEQRNGFIQSLKDDPSVSKEILAEAKKLNDAQAPKADLKFLKEIQNAFYWILHLPNLTEEQRNGFIQSLKDDPSVSKEILAEAKKLNDAQAPKADLKFLKEIQNAFYWILHLPNLTEEQRNGFIQSLKDDPSVSKEILAEAKKLNDAQAPK

SEQ ID NO: 97 - protein, 232 aa, synthetic construct
ADLKFLKEIQNAFYLILHLPNLTEEQRNGFIQSLKDDPSVSKEILAEAKKLNDAQAPKADLKFLKEIQNAFYLILHLPNLTEEQRNGFIQSLKDDPSVSKEILAEAKKLNDAQAPKADLKFLKEIQNAFYLILHLPNLTEEQRNGFIQSLKDDPSVSKEILAEAKKLNDAQAPKADLKFLKEIQNAFYLILHLPNLTEEQRNGFIQSLKDDPSVSKEILAEAKKLNDAQAPK

SEQ ID NO: 98 - protein, 232 aa, synthetic construct
ADYKFEKEIQNAFYIILHLPNLTEEQRNGFIQSLKDDPSVSKEILAEAKKLNDAQAPKADYKFEKEIQNAFYIILHLPNLTEEQRNGFIQSLKDDPSVSKEILAEAKKLNDAQAPKADYKFEKEIQNAFYIILHLPNLTEEQRNGFIQSLKDDPSVSKEILAEAKKLNDAQAPKADYKFEKEIQNAFYIILHLPNLTEEQRNGFIQSLKDDPSVSKEILAEAKKLNDAQAPK

SEQ ID NO: 99 - protein, 232 aa, synthetic construct
ADVKFLKEIQNAFYVILHLPNLTEEQRNGFIQSLKDDPSVSKEILAEAKKLNDAQAPKADVKFLKEIQNAFYVILHLPNLTEEQRNGFIQSLKDDPSVSKEILAEAKKLNDAQAPKADVKFLKEIQNAFYVILHLPNLTEEQRNGFIQSLKDDPSVSKEILAEAKKLNDAQAPKADVKFLKEIQNAFYVILHLPNLTEEQRNGFIQSLKDDPSVSKEILAEAKKLNDAQAPK

SEQ ID NO: 100 - protein, 232 aa, synthetic construct
ADVKFEKEIQNAFYFILHLPNLTEEQRNGFIQSLKDDPSVSKEILAEAKKLNDAQAPKADVKFEKEIQNAFYFILHLPNLTEEQRNGFIQSLKDDPSVSKEILAEAKKLNDAQAPKADVKFEKEIQNAFYFILHLPNLTEEQRNGFIQSLKDDPSVSKEILAEAKKLNDAQAPKADVKFEKEIQNAFYFILHLPNLTEEQRNGFIQSLKDDPSVSKEILAEAKKLNDAQAPK

SEQ ID NO: 101 - protein, 232 aa, synthetic construct
ADYKFEKEIQNAFYLILHLPNLTEEQRNGFIQSLKDDPSVSKEILAEAKKLNDAQAPKADYKFEKEIQNAFYLILHLPNLTEEQRNGFIQSLKDDPSVSKEILAEAKKLNDAQAPKADYKFEKEIQNAFYLILHLPNLTEEQRNGFIQSLKDDPSVSKEILAEAKKLNDAQAPKADYKFEKEIQNAFYLILHLPNLTEEQRNGFIQSLKDDPSVSKEILAEAKKLNDAQAPK

SEQ ID NO: 102 - protein, 232 aa, synthetic construct
ADLKFLKEFQNAFYIILHLPNLTEEQRNGFIQSLKDDPSVSKEILAEAKKLNDAQAPKADLKFLKEFQNAFYIILHLPNLTEEQRNGFIQSLKDDPSVSKEILAEAKKLNDAQAPKADLKFLKEFQNAFYIILHLPNLTEEQRNGFIQSLKDDPSVSKEILAEAKKLNDAQAPKADLKFLKEFQNAFYIILHLPNLTEEQRNGFIQSLKDDPSVSKEILAEAKKLNDAQAPK

SEQ ID NO: 103 - protein, 232 aa, synthetic construct
ADVKFEKEIQNAFYLILHLPNLTEEQRNGFIQSLKDDPSVSKEILAEAKKLNDAQAPKADVKFEKEIQNAFYLILHLPNLTEEQRNGFIQSLKDDPSVSKEILAEAKKLNDAQAPKADVKFEKEIQNAFYLILHLPNLTEEQRNGFIQSLKDDPSVSKEILAEAKKLNDAQAPKADVKFEKEIQNAFYLILHLPNLTEEQRNGFIQSLKDDPSVSKEILAEAKKLNDAQAPK

SEQ ID NO: 104 - protein, 232 aa, synthetic construct
ADVKFEKEIQNAFYIILHLPNLTEEQRNGFIQSLKDDPSVSKEILAEAKKLNDAQAPKADVKFEKEIQNAFYIILHLPNLTEEQRNGFIQSLKDDPSVSKEILAEAKKLNDAQAPKADVKFEKEIQNAFYIILHLPNLTEEQRNGFIQSLKDDPSVSKEILAEAKKLNDAQAPKADVKFEKEIQNAFYIILHLPNLTEEQRNGFIQSLKDDPSVSKEILAEAKKLNDAQAPK

SEQ ID NO: 105 - protein, 348 aa, synthetic construct
ADLKFLKEIQNAFYLILHLPNLTEEQRNGFIQSLKDDPSVSKEILAEAKKLNDAQAPKADLKFLKEIQNAFYLILHLPNLTEEQRNGFIQSLKDDPSVSKEILAEAKKLNDAQAPKADLKFLKEIQNAFYLILHLPNLTEEQRNGFIQSLKDDPSVSKEILAEAKKLNDAQAPKADLKFLKEIQNAFYLILHLPNLTEEQRNGFIQSLKDDPSVSKEILAEAKKLNDAQAPKADLKFLKEIQNAFYLILHLPNLTEEQRNGFIQSLKDDPSVSKEILAEAKKLNDAQAPKADLKFLKEIQNAFYLILHLPNLTEEQRNGFIQSLKDDPSVSKEILAEAKKLNDAQAPK

SEQ ID NO: 106 - protein, 348 aa, synthetic construct
ADLKFEKEIQNAFYIILHLPNLTEEQRNGFIQSLKDDPSVSKEILAEAKKLNDAQAPKADLKFEKEIQNAFYIILHLPNLTEEQRNGFIQSLKDDPSVSKEILAEAKKLNDAQAPKADLKFEKEIQNAFYIILHLPNLTEEQRNGFIQSLKDDPSVSKEILAEAKKLNDAQAPKADLKFEKEIQNAFYIILHLPNLTEEQRNGFIQSLKDDPSVSKEILAEAKKLNDAQAPKADLKFEKEIQNAFYIILHLPNLTEEQRNGFIQSLKDDPSVSKEILAEAKKLNDAQAPKADLKFEKEIQNAFYIILHLPNLTEEQRNGFIQSLKDDPSVSKEILAEAKKLNDAQAPK

SEQ ID NO: 107 - protein, 348 aa, synthetic construct
ADVKFLKEIQNAFYVILHLPNLTEEQRNGFIQSLKDDPSVSKEILAEAKKLNDAQAPKADVKFLKEIQNAFYVILHLPNLTEEQRNGFIQSLKDDPSVSKEILAEAKKLNDAQAPKADVKFLKEIQNAFYVILHLPNLTEEQRNGFIQSLKDDPSVSKEILAEAKKLNDAQAPKADVKFLKEIQNAFYVILHLPNLTEEQRNGFIQSLKDDPSVSKEILAEAKKLNDAQAPKADVKFLKEIQNAFYVILHLPNLTEEQRNGFIQSLKDDPSVSKEILAEAKKLNDAQAPKADVKFLKEIQNAFYVILHLPNLTEEQRNGFIQSLKDDPSVSKEILAEAKKLNDAQAPK

SEQ ID NO: 108 - protein, 348 aa, synthetic construct
ADLKFEKEFQNAFYLILHLPNLTEEQRNGFIQSLKDDPSVSKEILAEAKKLNDAQAPKADLKFEKEFQNAFYLILHLPNLTEEQRNGFIQSLKDDPSVSKEILAEAKKLNDAQAPKADLKFEKEFQNAFYLILHLPNLTEEQRNGFIQSLKDDPSVSKEILAEAKKLNDAQAPKADLKFEKEFQNAFYLILHLPNLTEEQRNGFIQSLKDDPSVSKEILAEAKKLNDAQAPKADLKFEKEFQNAFYLILHLPNLTEEQRNGFIQSLKDDPSVSKEILAEAKKLNDAQAPKADLKFEKEFQNAFYLILHLPNLTEEQRNGFIQSLKDDPSVSKEILAEAKKLNDAQAPK

SEQ ID NO: 109 - protein, 58 aa, synthetic construct
  MUTAGEN 3: note = X is G, A, V, L, I, Y or F
  MUTAGEN 6: note = X is G, A, S, T, L, I, V, E or D
  MUTAGEN 9: note = X is G, A, L, V, Y, S, I, R, F or M
  MUTAGEN 15: note = X is G, L, A, M, F, Y, I, S, T, W, V, D, E or R
ADXKFXKEXQNAFYXILHLPNLTEEQRNGFIQSLKDDPSVSKEILAEAKKLNDAQAPK